European Patent Application EP 4 763 972 A1, published June 24, 2026. Title: 一种Akkermansia muciniphila及其产品和应用. Applicant: 善恩康生物科技（苏州）有限公司. Application CN 2023110476140, filed August 18, 2023. The sequence listing filed with the application follows.

SEQUENCE LISTING (19 sequences)

SEQ ID NO: 1 - DNA, 1362 bp, Akkermansia muciniphila
  source 1..1362: mol_type = genomic DNA
aacgagagaattgctagcttgctaataattctctagtggcgcacgggtgagtaacacgtgagtaacctgcccccgagagcgggatagccctgggaaactgggattaataccgcatagtatcgaaagattaaagcagcaatgcgcttggggatgggctcgcggcctattagttagttggtgaggtaacggctcaccaaggcgatgacgggtagccggtctgagaggatgtccggccacactggaactgagacacggtccagacacctacgggtggcagcagtcgagaatcattcacaatgggggaaaccctgatggtgcgacgccgcgtgggggaatgaaggtcttcggattgtaaacccctgtcatgtgggagcaaattaaaaagatagtaccacaagaggaagagacggctaactctgtgccagcagccgcggtaatacagaggtctcaagcgttgttcggaatcactgggcgtaaagcgtgcgtaggctgtttcgtaagtcgtgtgtgaaaggcgcgggctcaacccgcggacggcacatgatactgcgagactagagtaatggagggggaaccggaattctcggtgtagcagtgaaatgcgtagatatcgagaggaacactcgtggcgaaggcgggttcctggacattaactgacgctgaggcacgaaggccaggggagcgaaagggattagatacccctgtagtcctggcagtaaacggtgcacgcttggtgtgcggggaatcgaccccctgcgtgccggagctaacgcgttaagcgtgccgcctggggagtacggtcgcaagattaaaactcaaagaaattgacggggacccgcacaagcggtggagtatgtggcttaattcgatgcaacgcgaagaaccttacctgggcttgacatgtaatgaacaacatgtgaaagcatgcgactcttcggaggcgttacacaggtgctgcatggccgtcgtcagctcgtgtcgtgagatgtttggttaagtccagcaacgagcgcaacccctgttgccagttaccagcacgtgaaggtggggactctggcgagactgcccagatcaactgggaggaaggtggggacgacgtcaggtcagtatggcccttatgcccagggctgcacacgtactacaatgcccagtacagagggggccgaagccgcgaggcggaggaaatcctaaaaactgggcccagttcggactgtaggctgcaacccgcctacacgaagccggaatcgctagtaatggcgcatcagctacggcgccgtgaatacgttcccgggtcttgtacacaccgcccgtcacatcatggaagccggtcgcacccgaagtatctgaagccaaccgcaagga

SEQ ID NO: 2 - DNA, 19 bp, synthetic construct
  source 1..19: mol_type = other DNA
agagtttgatcctggctca

SEQ ID NO: 3 - DNA, 19 bp, synthetic construct
  source 1..19: mol_type = other DNA
ggttaccttgttacgactt

SEQ ID NO: 4 - DNA, 20 bp, synthetic construct
  source 1..20: mol_type = other DNA
tgtcagtcatcgcccatgtg

SEQ ID NO: 5 - DNA, 21 bp, synthetic construct
  source 1..21: mol_type = other DNA
catccttgcgagtgtcagtga

SEQ ID NO: 6 - DNA, 20 bp, synthetic construct
  source 1..20: mol_type = other DNA
agaggggatttcgattccgc

SEQ ID NO: 7 - DNA, 23 bp, synthetic construct
  source 1..23: mol_type = other DNA
cctgtgggtaggatttcttgttc

SEQ ID NO: 8 - DNA, 21 bp, synthetic construct
  source 1..21: mol_type = other DNA
tggcatccccgaatatgatga

SEQ ID NO: 9 - DNA, 22 bp, synthetic construct
  source 1..22: mol_type = other DNA
tgacagtaggataggtcttccg

SEQ ID NO: 10 - DNA, 20 bp, synthetic construct
  source 1..20: mol_type = other DNA
actgccgggatggctactat

SEQ ID NO: 11 - DNA, 21 bp, synthetic construct
  source 1..21: mol_type = other DNA
tctggattcgctggctaatgg

SEQ ID NO: 12 - DNA, 21 bp, synthetic construct
  source 1..21: mol_type = other DNA
gacatcgcatcggctcttaga

SEQ ID NO: 13 - DNA, 21 bp, synthetic construct
  source 1..21: mol_type = other DNA
aacggtcacggtgtacttctg

SEQ ID NO: 14 - DNA, 21 bp, synthetic construct
  source 1..21: mol_type = other DNA
tcctggtacatcgagaccttg

SEQ ID NO: 15 - DNA, 21 bp, synthetic construct
  source 1..21: mol_type = other DNA
aagtccctttcgcagaaacag

SEQ ID NO: 16 - DNA, 20 bp, synthetic construct
  source 1..20: mol_type = other DNA
ccagtcacgcaccatctttg

SEQ ID NO: 17 - DNA, 23 bp, synthetic construct
  source 1..23: mol_type = other DNA
gtccatctcgtttctaaccaagt

SEQ ID NO: 18 - DNA, 20 bp, synthetic construct
  source 1..20: mol_type = other DNA
cccggagatacggattgcac

SEQ ID NO: 19 - DNA, 20 bp, synthetic construct
  source 1..20: mol_type = other DNA
gcctcgcggtaatcatttgc